European Patent Specification EP 3 481 958 B1, published April 1, 2026. Title: METHODS AND COMPOSITIONS FOR TREATMENT OF DISORDERS AND DISEASES INVOLVING RDH12. Applicant: The Trustees of the University of Pennsylvania. Application EP 17824989.2. The sequence listing filed with the application follows.

SEQUENCE LISTING (4 sequences)

SEQ ID NO: 1 - DNA, 949 bp, Homo sapiens
atgctggtcaccttgggactgctcacctccttcttctcgttcctgtatatggtagctccatccatcaggaagttctttgctggtggagtgtgtagaacaaatgtgcagcttcctggcaaggtagtggtgatcactggcgccaacacgggcattggcaaggagacggccagagagctcgctagccgaggagcccgagtctatattgcctgcagagatgtactgaagggggagtctgctgccagtgaaatccgagtggatacaaagaactcccaggtgctggtgcggaaattggacctatccgacaccaaatctatccgagcctttgctgagggctttctggcagaggaaaagcagctccatattctgatcaacaatgcgggagtaatgatgtgtccatattccaagacagctgatggctttgaaacccacctgggagtcaaccacctgggccacttcctcctcacctacctgctcctggagcggctaaaggtgtctgcccctgcacgggtggttaatgtgtcctcggtggctcaccacattggcaagattcccttccacgacctccagagcgagaagcgctacagcaggggttttgcctattgccacagcaagctggccaatgtgctttttactcgtgagctggccaagaggctccaaggcaccggggtcaccacctacgcagtgcacccaggcgtcgtccgctctgagctggtccggcactcctccctgctctgcctgctctggcggctcttctccccctttgtcaagacggcacgggagggggcgcagaccagcctgcactgcgccctggctgagggcctggagcccctgagtggcaagtacttcagtgactgcaagaggacctgggtgtctccaagggcccgaaataacaaaacagctgagcgcctatggaatgtcagctgtgagcttctaggaatccggtgggagt

SEQ ID NO: 2 - protein, 316 aa, Homo sapiens
MLVTLGLLTSFFSFLYMVAPSIRKFFAGGVCRTNVQLPGKVVVITGANTGIGKETARELASRGARVYIACRDVLKGESAASEIRVDTKNSQVLVRKLDLSDTKSIRAFAEGFLAEEKQLHILINNAGVMMCPYSKTADGFETHLGVNHLGHFLLTYLLLERLKVSAPARVVNVSSVAHHIGKIPFHDLQSEKRYSRGFAYCHSKLANVLFTRELAKRLQGTGVTTYAVHPGVVRSELVRHSSLLCLLWRLFSPFVKTAREGAQTSLHCALAEGLEPLSGKYFSDCKRTWVSPRARNNKTAERLWNVSCELLGIRWE

SEQ ID NO: 3 - DNA, 949 bp, Artificial Sequence
  Codon-optimized RDH12 DNA sequencel.
atgttggtcaccctcggactccttacctcatttttctccttcctgtacatggtcgccccgagcattagaaagttcttcgccggcggagtgtgtaggactaacgtgcagttgcccgggaaggtcgtggtgattactggcgccaacactggtatcggaaaggaaactgcgcgggaactggcgtccagaggtgcccgcgtgtacattgcatgccgcgacgtgctgaagggagaatccgccgcgtccgagatccgggtggacaccaaaaatagccaggtgctcgtgcggaagctggatctgtccgacaccaagtcaatcagggcctttgccgaggggttcctggctgaagagaagcagctccacattctgatcaacaacgccggggtcatgatgtgcccctactcaaagaccgcagacggcttcgaaacccacctgggcgtgaaccatctgggacacttcctgctgacctatctgctgctggagcgactgaaagtgtcggctcctgctcgggtcgtgaacgtgtccagcgtggcccatcacatcggaaagatcccattccacgatctccaatccgagaagcggtacagcaggggcttcgcgtactgtcactcgaagttggccaacgtgctctttacccgcgaactggccaagcggctgcagggcactggcgtgaccacttacgccgtgcaccctggtgtcgtgcggtccgagctggtccgccattcctctcttctgtgcctcctgtggagactcttctccccgttcgtcaagaccgcaagggaaggagcccaaacgagccttcactgtgccctggcggaaggactggagccgcttagcggaaagtacttctcggactgcaagcgcacctgggtgtcgcctagagctcggaacaacaagactgccgaacgcctctggaatgtgtcctgcgagctgctgggaatcagatgggagt

SEQ ID NO: 4 - protein, 316 aa, Artificial Sequence; identical to SEQ ID NO: 2
  Translated functional RDH12 protein sequence.